European Patent Specification EP 3 636 744 B1, published February 21, 2024. Title: LACTOBACILLUS CURVATUS WIKIM55 HAVING PROMOTING THE HAIR GROWTH. Applicant: Korea Food Research Institute. The sequence listing filed with the application follows.

SEQUENCE LISTING (1 sequence)

SEQ ID NO: 1 - DNA, 1449 bp, Lactobacillus curvatus WIKIM55
acatgcaagtcgaacgcactctcgttagattgaagaagcttgcttctgattgataacatttgagtgagtggcggacgggtgagtaacacgtgggtaacctgccctaaagtgggggataacatttggaaacagatgctaataccgcataaaacctagcaccgcatggtgcaaggttgaaagatggtttcggctatcactttaggatggacccgcggtgcattagttagttggtgaggtaaaggctcaccaagaccgtgatgcatagccgacctgagagggtaatcggccacactgggactgagacacggcccagactcctacgggaggcagcagtagggaatcttccacaatggacgaaagtctgatggagcaacgccgcgtgagtgaagaaggttttcggatcgtaaaactctgttgttggagaagaacgtatttgatagtaactgatcaggtagtgacggtatccaaccagaaagccacggctaactacgtgccagcagccgcggtaatacgtaggtggcaagcgttgtccggatttattgggcgtaaagcgagcgcaggcggtttcttaagtctgatgtgaaagccttcggctcaaccgaagaagtgcatcggaaactgggaaacttgagtgcagaagaggacagtggaactccatgtgtagcggtgaaatgcgtagatatatggaagaacaccagtggcgaaggcggctgtctggtctgtaactgacgctgaggctcgaaagcatgggtagcaaacaggattagataccctggtagtccatgccgtaaacgatgagtgctaggtgttggagggtttccgcccttcagtgccgcagctaacgcattaagcactccgcctggggagtacgaccgcaaggttgaaactcaaaggaattgacgggggcccgcacaagcggtggagcatgtggtttaattcgaagcaacgcgaagaaccttaccaggtcttgacatcctttgaccactctagagatagagctttcccttcggggacaaagtgacaggtggtgcatggttgtcgtcagctcgtgtcgtgagatgttgggttaagtcccgcaacgagcgcaacccttattactagttgccagcatttagttgggcactctagtgagactgccggtgacaaaccggaggaaggtggggacgacgtcaaatcatcatgccccttatgacctgggctacacacgtgctacaatggatggtacaacgagtcgcgagaccgcgaggtttagctaatctcttaaaaccattctcagttcggattgtaggctgcaactcgcctacatgaagccggaatcgctagtaatcgcggatcagcatgccgcggtgaatacgttcccgggccttgtacacaccgcccgtcacaccatgaagagtttgtaacacccaaagccgggtgaggtaaccttcgggagccagccgtctaagg